European Patent Application EP 4 141 129 A1, published March 1, 2023. Title: METHOD FOR DETECTING HBV GENOTYPE, OLIGONUCLEOTIDE AND KIT. Applicant: Leadway (HK) Limited. Application PCT/CN2021/089334. The sequence listing filed with the application follows.

SEQUENCE LISTING (21 sequences)

SEQ ID NO: 2 - DNA, 22 bp, (Artificial Sequence)
gattatcaaggtatgttgcccg

SEQ ID NO: 2 - DNA, 19 bp, (Artificial Sequence)
tgccttgagcaggagtcgt

SEQ ID NO: 3 - DNA, 18 bp, (Artificial Sequence)
acaacaacaaccagtacg

SEQ ID NO: 4 - DNA, 19 bp, (Artificial Sequence)
aacacccgtgtgtcttggc

SEQ ID NO: 5 - DNA, 21 bp, (Artificial Sequence)
taaccaggacaaattggagga

SEQ ID NO: 6 - DNA, 17 bp, (Artificial Sequence)
ccaaatctccagtcact

SEQ ID NO: 7 - DNA, 19 bp, (Artificial Sequence)
ctaggacccctgctcgtgt

SEQ ID NO: 8 - DNA, 23 bp, (Artificial Sequence)
gagagaagtccaccacgagtcta

SEQ ID NO: 9 - DNA, 23 bp, (Artificial Sequence)
caggcggggtttttcttgttgac

SEQ ID NO: 10 - DNA, 22 bp, (Artificial Sequence)
ctcgtggtggacttctctcaat

SEQ ID NO: 11 - DNA, 19 bp, (Artificial Sequence)
gttggggactgcgaatttt

SEQ ID NO: 12 - DNA, 15 bp, (Artificial Sequence)
cacccamgtgtcctg

SEQ ID NO: 13 - DNA, 22 bp, (Artificial Sequence)
ctcgtggtggacttctctcaat

SEQ ID NO: 14 - DNA, 19 bp, (Artificial Sequence)
gttggggactgcgaatttt

SEQ ID NO: 15 - DNA, 15 bp, (Artificial Sequence)
acacacggtagttcc

SEQ ID NO: 16 - DNA, 22 bp, (Artificial Sequence)
atttggagcttccgtggagtta

SEQ ID NO: 17 - DNA, 24 bp, (Artificial Sequence)
gcagtatggtgaggtgaacaatgt

SEQ ID NO: 18 - DNA, 28 bp, (Artificial Sequence)
ccttctattcgagatctcctcgacaccg

SEQ ID NO: 19 - DNA, 22 bp, (Artificial Sequence)
tgcaagaaggatcgttgaagct

SEQ ID NO: 20 - DNA, 21 bp, (Artificial Sequence)
caacagtctggcctttcagca

SEQ ID NO: 21 - DNA, 25 bp, (Artificial Sequence)
atgagggcaggccgctatgatggat